European Patent Application EP 4 595 983 A1, published August 6, 2025. Title: Nanoparticle. Applicant: BXTA NANOTHERAPY LIMITED. The sequence listing filed with the application follows.

SEQUENCE LISTING (7 sequences)

SEQ ID NO: 1 - protein, 14 aa, synthetic construct
  MOD_RES 14: note = C-terminal Amidation
RTLFKAHMGQKHRC

SEQ ID NO: 2 - protein, 14 aa, synthetic construct
  MOD_RES 1: note = N-terminal Palmitoyl Arginine
RTLFKAHMGQKHRC

SEQ ID NO: 3 - protein, 14 aa, synthetic construct
  MOD_RES 1: note = N-terminal Palmitoyl Arginine
  MOD_RES 14: note = C-terminal Amidation
RTLFKAHMGQKHRC

SEQ ID NO: 4 - protein, 17 aa, synthetic construct
CKKKKKKSEDEYPYVPN

SEQ ID NO: 5 - protein, 24 aa, synthetic construct
GCGLFHAIAHFIHGGWHGHHGWYG

SEQ ID NO: 6 - protein, 13 aa, synthetic construct
  MOD_RES 1: note = N-terminal Palmitoyl Arginine
  MOD_RES 13: note = C-terminal Amidation
RTLFKAHMGQKHR

SEQ ID NO: 7 - protein, 14 aa, synthetic construct
  MOD_RES 1: note = N-terminal Palmitoyl Threonine
  MOD_RES 14: note = C-terminal Amidation
TRFLAKMHQGHKRC